European Patent Application EP 4 686 760 A1, published February 4, 2026. Title: Sialyltransferases for the synthesis of sialylated glycans, glycoconjugates and glycoproteins. Applicant: Max-Planck-Gesellschaft zur Förderung der Wissenschaften e.V. Application EP. The sequence listing filed with the application follows.

SEQUENCE LISTING (20 sequences)

SEQ ID NO: 1 - protein, 407 aa, Shewanella halifaxensis
  source 1..407: note = beta-galactoside-alpha2,6-sialyltransferase
APTLELYIDNASLPTLHQLMHIIESYEENLTRTRFISWGRVSITDEQVRDMLNISTFPLVSNNTSQKLVDAVKSYAQSKNRLNIEIYSNTTHALKNIKPIISSLSGNPNVNIAEINLYDDGSAEYINLYNWKNTPNKIDALNADLLVMKDYVEGYSTQSPSYMSSRYNWHKLYDTEYHFLRADYLTIEPNLNDLRDYLGNSLEQMDWGKFEQLSKAKQQLFLSIVGFDKDSLEKSYANSPNKNFVFTGTTTWAGNETREFYAKQQINVINNAINETSPLYLGEEYDLFFKGHPRGGDINNMILNAFKDMINIPASISFEVLMMTGSLPDKVAGIASSLYFTIPAEKVDFIVFTSSDDITDREEALKSPLVQVMMKLGIVEKQAVQFWSDLPNCESGVCINNHHHHHH

SEQ ID NO: 2 - protein, 408 aa, Photobacterium sp.
  source 1..408: note = alpha-2,6-sialyltransferase
MHHHHHHAPSLEVYVDHASLPTLQQLMDIIKSEEENPTAQRYIAWGRIVPTDEQMKELNITSFALINNHTPADLVQEIVKQAQTKHRLNVKLSSNTAHSFDNLVPILKELNSFNNVTVTNIDLYDDGSAEYVNLYNWRDTLNKTDNLKIGKDYLEDVINGINEDTSNTGTSSVYNWQKLYPANYHFLRKDYLTLEPSLHELRDYIGDSLKQMQWDGFKKFNSKQQELFLSIVNFDKQKLQNEYNSSNLPNFVFTGTTVWAGNHEREYYAKQQINVINNAINESSPHYLGNSYDLFFKGHPGGGIINTLIMQNYPSMVDIPSKISFEVLMMTDMLPDAVAGIASSLYFTIPAEKIKFIVFTSTETITDRETALRSPLVQVMIKLGIVKEENVLFWADLPNCETGVCIAV

SEQ ID NO: 3 - protein, 389 aa, Photobacterium phosphoreum
  source 1..389: note = alpha-2,3-sialyltransferase
HHHHHHKHNNSDGNITKNKTIEVYVDRATLPTIQQMTQIINENSNNKKLISWSRYPINDETLLESINGSFFKNRPELIKSLDSMILTNEIKKVIINGNTLWAVDVVNIIKSIEALGKKTEIELNFYDDGSAEYVRLYDFSRLPESEQEYKISLSKDNIQSSINGTQPFDNSIENIYGFSQLYPTTYHMLRADIFETNLPLTSLKRVISNNIKQMKWDYFTTFNSQQKNKFYNFTGFNPEKIKEQYKASPHENFIFIGTNSGTATAEQQIDILTEAKKPDSPIITNSIQGLDLFFKGHPSATYNQQIIDAHNMIEIYNKIPFEALIMTDALPDAVGGMGSSVFFSLPNTVENKFIFYKSDTDIENNALIQVMIELNIVNRNDVKLISDLQ

SEQ ID NO: 4 - protein, 384 aa, Brevinema andersonii
  source 1..384: note = alpha-2,6-sialyltransferase
MFPSPHLVKIYISHATVPAMQFFSDAAKNPDILKLIYTPRFTNNFNAIDNIRKHDNIDSLLLNIKQILKKYPSVKIELHTQIHPFKMYSDVLRAIPTNRLFHVYVYDDGSEDYVNFYINKKTGRQKEVLKASDEAWQKFFSGESNLIGHRNMIAKYLPVTHYMLRPDYLDHSDMKIVKDAMTQNNAQIKKIDFDNLRMQLSELEKKRYFKYIGFNYKKIKKILCQSSNFSFVFTGSAVYDDPQRAQKFVEEQINMIKNVIQPEGILHKYLNGKTYDFFLKLHPHGGDSNKKTKNAFPDFPNIPNFIGYEALIVSGLIPDRTGGFLSSLYFNLPKEKIAFLVASVDKTEWDDPLVQVMIELGIIRESSIYFLSDLKLLNHHHHHH

SEQ ID NO: 5 - protein, 401 aa, Shewanella halifaxensis
  source 1..401: note = alpha-2,6-sialyltransferase
APTLELYIDNASLPTLHQLMHIIESYEENKTRTRFISWGRVSITDEQVRDMLNISTFPLDSNNTSQKLVDAVKSYAQSKNRLNIEIYSNTTHALKNIKPIISSLSGNPNVNIAEINLYDDGSAEYINLYNWKNTPNKIDALNADLDVMKDYVEGRSTQSPSDMSSRYNWHKLYDTEYHFLRADYLTREPNLNDLRDYLGNSLEQMDWGKFEQLSKAKQQLFLSIVGFDKDSLEKSYANSPNKNFVFTGTTTWAGNETREFYAKQQINVINNAINETSPLYLGEEYDLFFKGHPRGGDINNMILNAFKDMINIPASISFEVLMMTGSLPDKVAGIASSLYFTIPAEKVDFIVFTSSDDITDREEALKSPLVQVMMKLGIVEKQAVQFWSDLPNCESGVCINN

SEQ ID NO: 6 - protein, 390 aa, Photobacterium kishitanii
  source 1..390: note = alpha-2,3-sialyltransferase
MHHHHHHSNNNPDENVTKNKTIEVYVDRATLPTIQQMTQIINNKSDDQKLISWSRYPISNMGLLKSINATFFTNNSDLIKSLDSLILTDEIKKVIIHGNTLWAVDVVDIIRTIEDFGKSTEIELQFYDDGSAEYVQLYDFSKLPESEQEYRVSLSKDNIKASINGNQSFDNSVENIYGFSQIYPTTYNMLRMDVFNTNLPLNPLKSLMLNNIKQMKWDYFMHFNDHQKNQFYTFTGFNPEKIKAQYKESPNENFIFVGSNSGTATADQQIDIITEAKKPDSLIIPRSIQEYDLFFKGHPSATYNQQIIDAHNMTEIYNKIPFEALIMTDTLPDAVGGMGSSVFFSLPNKVENKFIFYKSDTDIDNNSLIQVMITLHIVSREDVKLISDIE

SEQ ID NO: 7 - protein, 411 aa, Glaesserella australis
  source 1..411: note = alpha-2,3-sialyltransferase
MNKEEYQKVEIYLDFATIPTLNYFFHFIENYQDKDTIRLFGLGRFKIPDSVIEQYPAGKIYFAKSEIDAQHHHHHHHEFKQLCFGVLKNIDQKMVLNLHVNLTHSFVILASLLDILFSLEERKCHSICLHLYDDGAEGPRQLYTLSQRSDLEELVAFHKNQMANLLHAGKATISVLGVFRYLWQEIFTTHYHLLDTKVLDLASLAPLKSEMINYHKMSFNHFHKFNQEQKRLFLTLLDLDTKYENQIIDLFKNNKTFVFTGTTMFDCDSNLLNFLENAHTQIIENMIYPEGKYYHQYDDYIFLYKGHPHAKELNKRILEKFNKLINIPEHLPFEVLYLLGLNPTKIGGFFSTSYFQVESDRIADVFFLSSSDPEKNKKYYVFSEQYDLMKVLLALDYVKEEQCHLINFNIK

SEQ ID NO: 8 - protein, 399 aa, Ursidibacter arcticus
  source 1..399: note = alpha-2,3-sialyltransferase
MEKFEIYIDFATIPTLNYFYHFIDNLNDKDTTRWFALSRFEIPENIINIFPKGKVITYKVVEHNIEKLVEDFKHTVYNCQSKLDIRLHINLFHSLEILKNIIFIYANNRDKFENFSFCFYDDGAEGAVTLYELSKLDEVNLVNSIKEHNEILNNLVKCQNVRVHNQLLFRYLWNNVIRTSYCLCNTSLLDKGCLPMLKKQMGNIELMNFNKFHSFSDYQKDMMASLLNIKTNDIHNIINLSKMYKSTVLLGTTVFNISEDSIPVLENIHFNAIKEMTLPEGRFFNNKNDHLFFYKGHPHAKELNNRIKENFEHLIIIPDHIAFETLLLLGFKLDSLVGFAGTILFGVPKDIISEQIFLTKSEEKYRNSYLFNQQYELSRSLLSLGHIKEENVHFFDDFL

SEQ ID NO: 9 - protein, 394 aa, Gallalistipes aquisgranensis
  source 1..394: note = alpha-2,3-sialyltransferase
MHHHHHHDKEEGFRPSWIAEGADFDSPDHYFYVTFGTMPTLYAGLHMLSHDKPSYVFYERTATFDAGKLPSHVTVCPYMGANDQQPQMREWMKNKIREIDRENPQAIFGLYVDDLRCRLGYDWFVAQGIDSSRVKVTMLSDGTGTYNNFYNYFNVPGTGEQNWKTYASQVEALDWSYPRGYATRSIGEFESWEWPYYLSTRPGYRLLLQDASLFETQDPYVQEQMPAMYLWSRTPYEMLADLTEEERKKFFEMASFDRDAFDAGFDASSKKNLVIIGTNGDGDNQRAYVQRLYDEYKDRYDLFFKPHPSDVTSADYETAFPGLTLLPGQMPFEIFVWSLIDKIDMIGGYPSTVYLTVPVEKVTFLFASGPDALIRPLNLIFAAAQDRVEWMQPE

SEQ ID NO: 10 - protein, 392 aa, Trichormus variabilis
  source 1..392: note = AGE family epimerase/isomerase
MGKNLQALAQLYKNALLNDVLPFWENYSLDSEGGYFTCLDRQGKVYDTDKFIWLQNRQVWTFSMLCNQLEKRENWLKIARNGAKFLAQHGRDDEGNWYFALTRGGEPLVQPYNIFSDCFAAMAFSQYALASGEEWSKDVAMQAYNNVLRRKDNPKGKYTKTYPGTRPMKALAVPMILANLTLEMEWLLPQETLENVLAATVQEVMGDFLDQERGLMYENVAPDGSHIDCFEGRLINPGHGIEAMWFIMDIARRKNDSKTINQAVDVVLNILNFAWDNEYGGLYYFMDAAGHPPQQLEWDQKLWWVHLESLVALAMGYRLTGREVCWEWYQKMHDYSWQHFADPEYGEWFGYLNRRGEVLLNLKGGKWKGCFHVPRALYLCWQQFEALSLQSA

SEQ ID NO: 11 - protein, 293 aa, Pasteurella multocida subsp. multocida str. Pm70
  source 1..293: note = N-acetylneuraminate lyase (NAL)
MKNLKGIFSALLVSFNADGSINEKGLRQIVRYNIDKMKVDGLYVGGSTGENFMLSTEEKKEIFRIAKDEAKDEIALIAQVGSVNLQEAIELGKYATELGYDSLSAVTPFYYKFSFPEIKHYYDSIIEATGNYMIVYSIPFLTGVNIGVEQFGELYKNPKVLGVKFTAGDFYLLERLKKAYPNHLIWAGFDEMMLPAASLGVDGAIGSTFNVNGVRARQIFELTQAGKLKEALEIQHVTNDLIEGILANGLYLTIKELLKLDGVEAGYCREPMTKELSPEKVAFAKELKAKYLS

SEQ ID NO: 12 - protein, 228 aa, Neisseria meningitidis
  source 1..228: note = N-acylneuraminate cytidylyltransferase (CSS)
MEKQNIAVILARQNSKGLPLKNLRKMNGISLLGHTINAAISSKCFDRIIVSTDGGLIAEEAKNFGVEVVLRPAELASDTASSISGVIHALETIGSNSGTVTLLQPTSPLRTGAHIREAFSLFDEKIKGSVVSACPMEHHPLKTLLQINNGEYAPMRHLSDLEQPRQQLPQAFRPNGAIYINDTASLIANNCFFIAPTKLYIMSHQDSIDIDTELDLQQAENILNHKES

SEQ ID NO: 13 - protein, 213 aa, Escherichia coli
  source 1..213: note = Uridine kinase (UDK)
MTDQSHQCVIIGIAGASASGKSLIASTLYRELREQVGDEHIGVIPEDCYYKDQSHLSMEERVKTNYDHPSAMDHSLLLEHLQALKRGSAIDLPVYSYVEHTRMKETVTVEPKKVIILEGILLLTDARLRDELNFSIFVDTPLDICLMRRIKRDVNERGRSMDSVMAQYQKTVRPMFLQFIEPSKQYADIIVPRGGKNRIAIDILKAKISQFFE

SEQ ID NO: 14 - protein, 202 aa, Arabidopsis thaliana [sequence omitted]

SEQ ID NO: 15 - protein, 301 aa, Ruegeria pomeroyi
  source 1..301: note = Polyphosphate:NDP phosphotransferase 3 (PPK3)
MNRNGSTKDPRRMTGAATGEISRYFNDKAPKDIRRAIEKADKDDILSTTYPYDAEMTAKDYRAQMEALQIELVKLQAWIKQSGARVALLFEGRDAAGKGGTIKRFRENLNPRGARVVALSKPTEAERSQWYFQRYIQHLPSAGELVFYDRSWYNRGVVEHVFGWCDEEQRERFFRQVMPFEHDLVDDGIHLFKFWLNVGRAEQLRRFHDRERDPLKQWKLSPVDIAGLDKWEAYTTAISQTLTRSHSDRAPWTVIRSDDKKRARLAAIRTVLSGIDYDNKDRAAVGQPDAAICGGPDIWDA

SEQ ID NO: 16 - protein, 175 aa, Pasteurella multocida subsp. multocida str. Pm70
  source 1..175: note = Inorganic pyrophosphatase (PPA)
MGLETVPAGKALPDDIYVVIEIPANSDPIKYEVDKESGALFVDRFMATAMFYPANYGYVNNTLSLDGDPVDVLVPTPYPLQPGSVIRCRPVGVLKMTDEAGSDAKVVAVPHSKLTKEYDHIKDVNDLPALLKAQIQHFFESYKALEAGKWVKVDGWEGVDAARQEILDSFERAKK

SEQ ID NO: 17 - protein, 505 aa, Pseudomonas aeruginosa
  source 1..505: note = Polyphosphate: AMP phosphotransferase (2D-PPK2)
MVFESAEVGHSIDKDTYEKAVIELREALLEAQFELKQQARFPVIILINGIEGAGKGETVKLLNEWMDPRLIEVQSFLRPSDEELERPPQWRFWRRLPPKGRTGIFFGNWYSQMLYARVEGHIKEAKLDQAIDAAERFERMLCDEGALLFKFWFHLSKKQLKERLKALEKDPQHSWKLSPLDWKQSEVYDRFVHYGERVLRRTSRDYAPWYVVEGADERYRALTVGRILLEGLQAALATKERAKRQPHAAPLVSSLDNRGLLDSLDLGQYLDKDAYKEQLAAEQARLAGLIRDKRFRQHSLVAVFEGNDAAGKGGAIRRVTDALDPRQYHIVPIAAPTEEERAQPYLWRFWRHIPARRQFTIFDRSWYGRVLVERIEGFCAPADWLRAYGEINDFEEQLSEYGIIVVKFWLAIDKQTQMERFKEREKTPYKRYKITEEDWRNRDKWDQYVDAVGDMVDRTSTEIAPWTLVEANDKRFARVKVLRTINDAIEAAYKKDKLEHHHHHH

SEQ ID NO: 18 - protein, 324 aa, Pseudomonas aeruginosa
  source 1..324: note = Polyphosphate:ADP phosphotransferase (1D-PPK2)
MGSSHHHHHHSSGLVPRGSHMDSYGDTSGRIGRDWLDRHDEELEQELLDDELNLDELFGPEQEDAPGELSRRRYFRELFRLQRELVKLQNWVVHTGHKVVILFEGRDAAGKGGVIKRITQRLNPRVCRVAALPAPNDREQTQWYFQRYVSHLPAGGEIVLFDRSWYNRAGVERVMGFCNDEQYEEFFRSVPEFEKMLARSGIQLLKYWFSISDAEQHLRFLSRIHDPLKQWKLSPMDLESRRRWEAYTKAKETMLERTHIPEAPWWVVQADDKKRARLNCIHHLLQQMPYREVPQPPVHLPERLRHADYVRHPTPGEIIVPEVY

SEQ ID NO: 19 - DNA, 5369 bp, synthetic construct
  source 1..5369: mol_type = other DNA; note = Vector Sequence pET-28a(+)
atccggatatagttcctcctttcagcaaaaaacccctcaagacccgtttagaggccccaaggggttatgctagttattgctcagcggtggcagcagccaactcagcttcctttcgggctttgttagcagccggatctcagtggtggtggtggtggtgctcgagtgcggccgcaagcttgtcgacggagctcgaattcggatccgcgacccatttgctgtccaccagtcatgctagccatatggctgccgcgcggcaccaggccgctgctgtgatgatgatgatgatggctgctgcccatggtatatctccttcttaaagttaaacaaaattatttctagaggggaattgttatccgctcacaattcccctatagtgagtcgtattaatttcgcgggatcgagatctcgatcctctacgccggacgcatcgtggccggcatcaccggcgccacaggtgcggttgctggcgcctatatcgccgacatcaccgatggggaagatcgggctcgccacttcgggctcatgagcgcttgtttcggcgtgggtatggtggcaggccccgtggccgggggactgttgggcgccatctccttgcatgcaccattccttgcggcggcggtgctcaacggcctcaacctactactgggctgcttcctaatgcaggagtcgcataagggagagcgtcgagatcccggacaccatcgaatggcgcaaaacctttcgcggtatggcatgatagcgcccggaagagagtcaattcagggtggtgaatgtgaaaccagtaacgttatacgatgtcgcagagtatgccggtgtctcttatcagaccgtttcccgcgtggtgaaccaggccagccacgtttctgcgaaaacgcgggaaaaagtggaagcggcgatggcggagctgaattacattcccaaccgcgtggcacaacaactggcgggcaaacagtcgttgctgattggcgttgccacctccagtctggccctgcacgcgccgtcgcaaattgtcgcggcgattaaatctcgcgccgatcaactgggtgccagcgtggtggtgtcgatggtagaacgaagcggcgtcgaagcctgtaaagcggcggtgcacaatcttctcgcgcaacgcgtcagtgggctgatcattaactatccgctggatgaccaggatgccattgctgtggaagctgcctgcactaatgttccggcgttatttcttgatgtctctgaccagacacccatcaacagtattattttctcccatgaagacggtacgcgactgggcgtggagcatctggtcgcattgggtcaccagcaaatcgcgctgttagcgggcccattaagttctgtctcggcgcgtctgcgtctggctggctggcataaatatctcactcgcaatcaaattcagccgatagcggaacgggaaggcgactggagtgccatgtccggttttcaacaaaccatgcaaatgctgaatgagggcatcgttcccactgcgatgctggttgccaacgatcagatggcgctgggcgcaatgcgcgccattaccgagtccgggctgcgcgttggtgcggatatctcggtagtgggatacgacgataccgaagacagctcatgttatatcccgccgttaaccaccatcaaacaggattttcgcctgctggggcaaaccagcgtggaccgcttgctgcaactctctcagggccaggcggtgaagggcaatcagctgttgcccgtctcactggtgaaaagaaaaaccaccctggcgcccaatacgcaaaccgcctctccccgcgcgttggccgattcattaatgcagctggcacgacaggtttcccgactggaaagcgggcagtgagcgcaacgcaattaatgtaagttagctcactcattaggcaccgggatctcgaccgatgcccttgagagccttcaacccagtcagctccttccggtgggcgcggggcatgactatcgtcgccgcacttatgactgtcttctttatcatgcaactcgtaggacaggtgccggcagcgctctgggtcattttcggcgaggaccgctttcgctggagcgcgacgatgatcggcctgtcgcttgcggtattcggaatcttgcacgccctcgctcaagccttcgtcactggtcccgccaccaaacgtttcggcgagaagcaggccattatcgccggcatggcggccccacgggtgcgcatgatcgtgctcctgtcgttgaggacccggctaggctggcggggttgccttactggttagcagaatgaatcaccgatacgcgagcgaacgtgaagcgactgctgctgcaaaacgtctgcgacctgagcaacaacatgaatggtcttcggtttccgtgtttcgtaaagtctggaaacgcggaagtcagcgccctgcaccattatgttccggatctgcatcgcaggatgctgctggctaccctgtggaacacctacatctgtattaacgaagcgctggcattgaccctgagtgatttttctctggtcccgccgcatccataccgccagttgtttaccctcacaacgttccagtaaccgggcatgttcatcatcagtaacccgtatcgtgagcatcctctctcgtttcatcggtatcattacccccatgaacagaaatcccccttacacggaggcatcagtgaccaaacaggaaaaaaccgcccttaacatggcccgctttatcagaagccagacattaacgcttctggagaaactcaacgagctggacgcggatgaacaggcagacatctgtgaatcgcttcacgaccacgctgatgagctttaccgcagctgcctcgcgcgtttcggtgatgacggtgaaaacctctgacacatgcagctcccggagacggtcacagcttgtctgtaagcggatgccgggagcagacaagcccgtcagggcgcgtcagcgggtgttggcgggtgtcggggcgcagccatgacccagtcacgtagcgatagcggagtgtatactggcttaactatgcggcatcagagcagattgtactgagagtgcaccatatatgcggtgtgaaataccgcacagatgcgtaaggagaaaataccgcatcaggcgctcttccgcttcctcgctcactgactcgctgcgctcggtcgttcggctgcggcgagcggtatcagctcactcaaaggcggtaatacggttatccacagaatcaggggataacgcaggaaagaacatgtgagcaaaaggccagcaaaaggccaggaaccgtaaaaaggccgcgttgctggcgtttttccataggctccgcccccctgacgagcatcacaaaaatcgacgctcaagtcagaggtggcgaaacccgacaggactataaagataccaggcgtttccccctggaagctccctcgtgcgctctcctgttccgaccctgccgcttaccggatacctgtccgcctttctcccttcgggaagcgtggcgctttctcatagctcacgctgtaggtatctcagttcggtgtaggtcgttcgctccaagctgggctgtgtgcacgaaccccccgttcagcccgaccgctgcgccttatccggtaactatcgtcttgagtccaacccggtaagacacgacttatcgccactggcagcagccactggtaacaggattagcagagcgaggtatgtaggcggtgctacagagttcttgaagtggtggcctaactacggctacactagaaggacagtatttggtatctgcgctctgctgaagccagttaccttcggaaaaagagttggtagctcttgatccggcaaacaaaccaccgctggtagcggtggtttttttgtttgcaagcagcagattacgcgcagaaaaaaaggatctcaagaagatcctttgatcttttctacggggtctgacgctcagtggaacgaaaactcacgttaagggattttggtcatgaacaataaaactgtctgcttacataaacagtaatacaaggggtgttatgagccatattcaacgggaaacgtcttgctctaggccgcgattaaattccaacatggatgctgatttatatgggtataaatgggctcgcgataatgtcgggcaatcaggtgcgacaatctatcgattgtatgggaagcccgatgcgccagagttgtttctgaaacatggcaaaggtagcgttgccaatgatgttacagatgagatggtcagactaaactggctgacggaatttatgcctcttccgaccatcaagcattttatccgtactcctgatgatgcatggttactcaccactgcgatccccgggaaaacagcattccaggtattagaagaatatcctgattcaggtgaaaatattgttgatgcgctggcagtgttcctgcgccggttgcattcgattcctgtttgtaattgtccttttaacagcgatcgcgtatttcgtctcgctcaggcgcaatcacgaatgaataacggtttggttgatgcgagtgattttgatgacgagcgtaatggctggcctgttgaacaagtctggaaagaaatgcataaacttttgccattctcaccggattcagtcgtcactcatggtgatttctcacttgataaccttatttttgacgaggggaaattaataggttgtattgatgttggacgagtcggaatcgcagaccgataccaggatcttgccatcctatggaactgcctcggtgagttttctccttcattacagaaacggctttttcaaaaatatggtattgataatcctgatatgaataaattgcagtttcatttgatgctcgatgagtttttctaagaattaattcatgagcggatacatatttgaatgtatttagaaaaataaacaaataggggttccgcgcacatttccccgaaaagtgccacctgaaattgtaaacgttaatattttgttaaaattcgcgttaaatttttgttaaatcagctcattttttaaccaataggccgaaatcggcaaaatcccttataaatcaaaagaatagaccgagatagggttgagtgttgttccagtttggaacaagagtccactattaaagaacgtggactccaacgtcaaagggcgaaaaaccgtctatcagggcgatggcccactacgtgaaccatcaccctaatcaagttttttggggtcgaggtgccgtaaagcactaaatcggaaccctaaagggagcccccgatttagagcttgacggggaaagccggcgaacgtggcgagaaaggaagggaagaaagcgaaaggagcgggcgctagggcgctggcaagtgtagcggtcacgctgcgcgtaaccaccacacccgccgcgcttaatgcgccgctacagggcgcgtcccattcgcca

SEQ ID NO: 20 - DNA, 5493 bp, synthetic construct
  source 1..5493: mol_type = other DNA; note = Vector Sequence pET-22b(+)
atccggatatagttcctcctttcagcaaaaaacccctcaagacccgtttagaggccccaaggggttatgctagttattgctcagcggtggcagcagccaactcagcttcctttcgggctttgttagcagccggatctcagtggtggtggtggtggtgctcgagtgcggccgcaagcttgtcgacggagctcgaattcggatccgaattaattccgatatccatggccatcgccggctgggcagcgaggagcagcagaccagcagcagcggtcggcagcaggtatttcatatgtatatctccttcttaaagttaaacaaaattatttctagaggggaattgttatccgctcacaattcccctatagtgagtcgtattaatttcgcgggatcgagatctcgatcctctacgccggacgcatcgtggccggcatcaccggcgccacaggtgcggttgctggcgcctatatcgccgacatcaccgatggggaagatcgggctcgccacttcgggctcatgagcgcttgtttcggcgtgggtatggtggcaggccccgtggccgggggactgttgggcgccatctccttgcatgcaccattccttgcggcggcggtgctcaacggcctcaacctactactgggctgcttcctaatgcaggagtcgcataagggagagcgtcgagatcccggacaccatcgaatggcgcaaaacctttcgcggtatggcatgatagcgcccggaagagagtcaattcagggtggtgaatgtgaaaccagtaacgttatacgatgtcgcagagtatgccggtgtctcttatcagaccgtttcccgcgtggtgaaccaggccagccacgtttctgcgaaaacgcgggaaaaagtggaagcggcgatggcggagctgaattacattcccaaccgcgtggcacaacaactggcgggcaaacagtcgttgctgattggcgttgccacctccagtctggccctgcacgcgccgtcgcaaattgtcgcggcgattaaatctcgcgccgatcaactgggtgccagcgtggtggtgtcgatggtagaacgaagcggcgtcgaagcctgtaaagcggcggtgcacaatcttctcgcgcaacgcgtcagtgggctgatcattaactatccgctggatgaccaggatgccattgctgtggaagctgcctgcactaatgttccggcgttatttcttgatgtctctgaccagacacccatcaacagtattattttctcccatgaagacggtacgcgactgggcgtggagcatctggtcgcattgggtcaccagcaaatcgcgctgttagcgggcccattaagttctgtctcggcgcgtctgcgtctggctggctggcataaatatctcactcgcaatcaaattcagccgatagcggaacgggaaggcgactggagtgccatgtccggttttcaacaaaccatgcaaatgctgaatgagggcatcgttcccactgcgatgctggttgccaacgatcagatggcgctgggcgcaatgcgcgccattaccgagtccgggctgcgcgttggtgcggatatctcggtagtgggatacgacgataccgaagacagctcatgttatatcccgccgttaaccaccatcaaacaggattttcgcctgctggggcaaaccagcgtggaccgcttgctgcaactctctcagggccaggcggtgaagggcaatcagctgttgcccgtctcactggtgaaaagaaaaaccaccctggcgcccaatacgcaaaccgcctctccccgcgcgttggccgattcattaatgcagctggcacgacaggtttcccgactggaaagcgggcagtgagcgcaacgcaattaatgtaagttagctcactcattaggcaccgggatctcgaccgatgcccttgagagccttcaacccagtcagctccttccggtgggcgcggggcatgactatcgtcgccgcacttatgactgtcttctttatcatgcaactcgtaggacaggtgccggcagcgctctgggtcattttcggcgaggaccgctttcgctggagcgcgacgatgatcggcctgtcgcttgcggtattcggaatcttgcacgccctcgctcaagccttcgtcactggtcccgccaccaaacgtttcggcgagaagcaggccattatcgccggcatggcggccccacgggtgcgcatgatcgtgctcctgtcgttgaggacccggctaggctggcggggttgccttactggttagcagaatgaatcaccgatacgcgagcgaacgtgaagcgactgctgctgcaaaacgtctgcgacctgagcaacaacatgaatggtcttcggtttccgtgtttcgtaaagtctggaaacgcggaagtcagcgccctgcaccattatgttccggatctgcatcgcaggatgctgctggctaccctgtggaacacctacatctgtattaacgaagcgctggcattgaccctgagtgatttttctctggtcccgccgcatccataccgccagttgtttaccctcacaacgttccagtaaccgggcatgttcatcatcagtaacccgtatcgtgagcatcctctctcgtttcatcggtatcattacccccatgaacagaaatcccccttacacggaggcatcagtgaccaaacaggaaaaaaccgcccttaacatggcccgctttatcagaagccagacattaacgcttctggagaaactcaacgagctggacgcggatgaacaggcagacatctgtgaatcgcttcacgaccacgctgatgagctttaccgcagctgcctcgcgcgtttcggtgatgacggtgaaaacctctgacacatgcagctcccggagacggtcacagcttgtctgtaagcggatgccgggagcagacaagcccgtcagggcgcgtcagcgggtgttggcgggtgtcggggcgcagccatgacccagtcacgtagcgatagcggagtgtatactggcttaactatgcggcatcagagcagattgtactgagagtgcaccatatatgcggtgtgaaataccgcacagatgcgtaaggagaaaataccgcatcaggcgctcttccgcttcctcgctcactgactcgctgcgctcggtcgttcggctgcggcgagcggtatcagctcactcaaaggcggtaatacggttatccacagaatcaggggataacgcaggaaagaacatgtgagcaaaaggccagcaaaaggccaggaaccgtaaaaaggccgcgttgctggcgtttttccataggctccgcccccctgacgagcatcacaaaaatcgacgctcaagtcagaggtggcgaaacccgacaggactataaagataccaggcgtttccccctggaagctccctcgtgcgctctcctgttccgaccctgccgcttaccggatacctgtccgcctttctcccttcgggaagcgtggcgctttctcatagctcacgctgtaggtatctcagttcggtgtaggtcgttcgctccaagctgggctgtgtgcacgaaccccccgttcagcccgaccgctgcgccttatccggtaactatcgtcttgagtccaacccggtaagacacgacttatcgccactggcagcagccactggtaacaggattagcagagcgaggtatgtaggcggtgctacagagttcttgaagtggtggcctaactacggctacactagaaggacagtatttggtatctgcgctctgctgaagccagttaccttcggaaaaagagttggtagctcttgatccggcaaacaaaccaccgctggtagcggtggtttttttgtttgcaagcagcagattacgcgcagaaaaaaaggatctcaagaagatcctttgatcttttctacggggtctgacgctcagtggaacgaaaactcacgttaagggattttggtcatgagattatcaaaaaggatcttcacctagatccttttaaattaaaaatgaagttttaaatcaatctaaagtatatatgagtaaacttggtctgacagttaccaatgcttaatcagtgaggcacctatctcagcgatctgtctatttcgttcatccatagttgcctgactccccgtcgtgtagataactacgatacgggagggcttaccatctggccccagtgctgcaatgataccgcgagacccacgctcaccggctccagatttatcagcaataaaccagccagccggaagggccgagcgcagaagtggtcctgcaactttatccgcctccatccagtctattaattgttgccgggaagctagagtaagtagttcgccagttaatagtttgcgcaacgttgttgccattgctgcaggcatcgtggtgtcacgctcgtcgtttggtatggcttcattcagctccggttcccaacgatcaaggcgagttacatgatcccccatgttgtgcaaaaaagcggttagctccttcggtcctccgatcgttgtcagaagtaagttggccgcagtgttatcactcatggttatggcagcactgcataattctcttactgtcatgccatccgtaagatgcttttctgtgactggtgagtactcaaccaagtcattctgagaatagtgtatgcggcgaccgagttgctcttgcccggcgtcaatacgggataataccgcgccacatagcagaactttaaaagtgctcatcattggaaaacgttcttcggggcgaaaactctcaaggatcttaccgctgttgagatccagttcgatgtaacccactcgtgcacccaactgatcttcagcatcttttactttcaccagcgtttctgggtgagcaaaaacaggaaggcaaaatgccgcaaaaaagggaataagggcgacacggaaatgttgaatactcatactcttcctttttcaatattattgaagcatttatcagggttattgtctcatgagcggatacatatttgaatgtatttagaaaaataaacaaataggggttccgcgcacatttccccgaaaagtgccacctgaaattgtaaacgttaatattttgttaaaattcgcgttaaatttttgttaaatcagctcattttttaaccaataggccgaaatcggcaaaatcccttataaatcaaaagaatagaccgagatagggttgagtgttgttccagtttggaacaagagtccactattaaagaacgtggactccaacgtcaaagggcgaaaaaccgtctatcagggcgatggcccactacgtgaaccatcaccctaatcaagttttttggggtcgaggtgccgtaaagcactaaatcggaaccctaaagggagcccccgatttagagcttgacggggaaagccggcgaacgtggcgagaaaggaagggaagaaagcgaaaggagcgggcgctagggcgctggcaagtgtagcggtcacgctgcgcgtaaccaccacacccgccgcgcttaatgcgccgctacagggcgcgtcccattcgcca